European Patent Specification EP 4 056 717 B1, published May 1, 2024. Title: Composition for detecting Q fever and method of diagnosing Q fever using the same. Applicant: Industry Academic Cooperation Foundation of Chosun University. The sequence listing filed with the application follows.

SEQUENCE LISTING (10 sequences)

SEQ ID NO: 1 - DNA, 19 bp, Artificial Sequence
  Coxi IS1111 144F primer
gtggggtaaagtgatctac

SEQ ID NO: 2 - DNA, 18 bp, Artificial Sequence
  Coxi IS1111 275R primer
cccataaacgtccgatac

SEQ ID NO: 3 - DNA, 20 bp, Artificial Sequence
  Coxi IS1111 241P probe
cacacgcttccatcaccacg

SEQ ID NO: 4 - DNA, 18 bp, Artificial Sequence
  Coxi IS1111 130F primer
tgtggaattgatgagtgg

SEQ ID NO: 5 - DNA, 18 bp, Artificial Sequence
  Coxi IS1111 93F primer
actgggtgttgatattgc

SEQ ID NO: 6 - DNA, 25 bp, Artificial Sequence
  Coxi IS1111 72F primer
gtccatgaaagatattaaaatactg

SEQ ID NO: 7 - DNA, 18 bp, Artificial Sequence
  Coxi IS1111 266R primer
gtccgataccaatggttc

SEQ ID NO: 8 - DNA, 19 bp, Artificial Sequence
  Coxi IS1111 144F primer
gtggggtaaagtgatctac

SEQ ID NO: 9 - DNA, 25 bp, Artificial Sequence
  Coxi IS1111 182P primer
ctcagtatgtatccaccgtagccag

SEQ ID NO: 10 - DNA, 1095 bp, Artificial Sequence
  Coxiella burnetii IS1111 DNA sequence
atggacccaccccttaaagacggcgtcataatgcgccaacatagaatttctattttcaaaaaaaggagaaggtccatgaaagatattaaaatactgggtgttgatattgcaaaagatgtttttcaactgtgtggaattgatgagtggggtaaagtgatctacacgagacgggttaagcgtgctcagtatgtatccaccgtagccagtcttaaggtgggctgcgtggtgatggaagcgtgtggaggagcgaaccattggtatcggacgtttatggggatgggtatcccaacgcagttgatcagtccgcagcacgtcaaaccgtatgtcaaaagtaacaagaatgatcgtaacgatgcgcaggcgatagctgaagcggcttcccgcgcctcgatgcggtttgtgcagggtaaaacggtggaacaacaagacgttcaagcgctgttaaagatacgcgatcgtttagtcaaaagccgcacggcgctgatcaatgagattcgggggttgttgcaagaatacggactcacgatggcgcgtggtgccaagcgattttatgaagagctcccgttgattttagcgagcgaagcggtgggattaacaccgcggatgaaacgggtgttgaattgtttgtataccgaattgttgaaccgggacgaagcgattggtgattacgaggaggaattaaaagcggtggcaaaagccaatgaggattgtcaacgggtacagagcatcccgggggtgggttatttaacggcgctctcggtttatgcgagcgtgggtgacattcatcaatttcatcgttcccggcagttgtcggcgtttattgggttggtccctcgacaacattcgagtgggaataaggaggtgttgttggggattagtaaacgcggcaatgtgatgttaaggacgttattgattcatggcgcccgtgcgctattgcgtcatgtaaaaaataaaacggataaaaagagtctgtggttaaaagcactcattgagcgccgcggaatgaatcgcgcttgtgtggcgttagcgaataaaaatgcgccgatcatttgggcgcttttaacacgccaagaaacgtatcgctgtggcgcctaa